European Patent Specification EP 3 617 321 B1, published October 23, 2024. Title: METHODS AND COMPOSITIONS FOR THE EXTRACTION AND AMPLIFICATION OF NUCLEIC ACID FROM A SAMPLE. Applicant: Sequenom, Inc. The sequence listing filed with the application follows.

SEQUENCE LISTING (5 sequences)

SEQ ID NO: 1 - DNA, 20 bp, Artificial Sequence
  /note="Description of artificial sequence: 5' adapter"
acacggcgcacgcctccacg

SEQ ID NO: 2 - DNA, 12 bp, Artificial Sequence
  /note="Description of artificial sequence: 3' adapter"
cgtggaggcgtg

SEQ ID NO: 3 - DNA, 20 bp, Artificial Sequence
  /note="Description of artificial sequence: 5' adapter"
acacggcgcacgcctccacg

SEQ ID NO: 4 - DNA, 12 bp, Artificial Sequence
  /note="Description of artificial sequence: 3' adapter"
gtgcggaggtgc

SEQ ID NO: 5 - DNA, 12 bp, Artificial Sequence
  /note="Description of artificial sequence: SSGA13dd3' ;13 nucleobases with a dideoxy-nucleotide at its 3' position."
cgtggaggcgtg